European Patent Application EP 4 814 108 A1, published September 30, 2026. Title: Salicylic acid-producing Hydrogenophilus bacterium transformant. Applicant: 株式会社ＣＯ２資源化研究所. The sequence listing filed with the application follows.

SEQUENCE LISTING (22 sequences)

SEQ ID NO: 1 - DNA, 5219 bp, synthetic construct
  source 1..5219: mol_type = other DNA
cccatcgactgcacggtgcaccaatgcttctggcgtcaggcagccatcggaagctgtggtatggctgtgcaggtcgtaaatcactgcataattcgtgtcgctcaaggcgcactcccgttctggataatgttttttgcgccgacatcataacggttctggcaaatattctgaaatgagctgttgacaattaatcatcggctcgtataatgtgtggaattgtgagcggataacaatttcacacaggaaacaggccagttaggcctgctagcagatctggaggagaaacgcatatgctgatatcggatccgaattcgagctccgtcgacaagcttgcggccgcactgcagcaccatcaccaccatcattgataagatccggctgctaacaaagcccgaaaggaagctgagttggctgctgccaccgctgagcaataactcgaggccaatgaggccttcaaataaaacgaaaggctcagtcgaaagactgggcctttcgttttatctgttgtttgtcggtgaacgctctcctgagtaggacaaatccgccgggagcggatttgaacgttgcgaagcaacggcccggagggtggcgggcaggacgcccgccataaactgccaggcatcaaattaagcagaaggccatcctgacggatggcctttttgcgtttctacaaactccgcggatctaggtgaagatcctttttgataatctcatgaccaaaatcccttaacgtgagttttcgttccactgagcgtcagaccccgtagaaaagatcaaaggatcttcttgagatcctttttttctgcgcgtaatctgctgcttgcaaacaaaaaaaccaccgctaccagcggtggtttgtttgccggatcaagagctaccaactctttttccgaaggtaactggcttcagcagagcgcagataccaaatactgtccttctagtgtagccgtagttaggccaccacttcaagaactctgtagcaccgcctacatacctcgctctgctaatcctgttaccagtggctgctgccagtggcgataagtcgtgtcttaccgggttggactcaagacgatagttaccggataaggcgcagcggtcgggctgaacggggggttcgtgcacacagcccagcttggagcgaacgacctacaccgaactgagatacctacagcgtgagctatgagaaagcgccacgcttcccgaagggagaaaggcggacaggtatccggtaagcggcagggtcggaacaggagagcgcacgagggagcttccagggggaaacgcctggtatctttatagtcctgtcgggtttcgccacctctgacttgagcgtcgatttttgtgatgctcgtcaggggggcggagcctatggaaaaacgccagcaacgcggcctttttacggttcctggccttttgctggccgcggacgtagaaagccagtccgcagaaacggtgctgaccccggatgaatgtcagctactgggctatctggacaagggaaaacgcaagcgcaaagagaaagcaggtagcttgcagtgggcttacatggcgatagctagactgggcggttttatggacagcaagcgaaccggaattgccagctggggcgccctctggtaaggttgggaagccctgcaaagtaaactggatggctttcttgccgccaaggatctgatggcgcaggggatcaagatccgatcaagagaggccactaaggcccaggatgaggatcgtttcgcatgattgaacaagatggattgcacgcaggttctccggccgcttgggtggagaggctattcggctatgactgggcacaacagacaatcggctgctctgatgccgccgtgttccggctgtcagcgcaggggcgcccggttctttttgtcaagaccgacctgtccggtgccctgaatgaactacaggacgaggcagcgcggctatcgtggctggccacgacgggcgttccttgcgcagctgtgctcgacgttgtcactgaagcgggaagggactggctgctattgggcgaagtgccggggcaggatctcctgtcatctcaccttgctcctgccgagaaagtatccatcatggctgatgcaatgcggcggctgcatacgcttgatccggctacctgcccattcgaccaccaagcgaaacatcgcatcgagcgagcacgtactcggatggaagccggtcttgtcgatcaggatgatctggacgaagagcatcaggggctcgcgccagccgaactgttcgccaggctcaaggcgcgtatgcccgacggcgaggatctcgtcgtgactcatggcgatgcctgcttgccgaatatcatggtggaaaatggccgcttttctggattcatcgactgtggccggctgggtgtggcggaccgctatcaggacatagcgttggctacccgtgatattgctgaagagcttggcggcgaatgggctgaccgcttcctcgtgctttacggtatcgccgctcccgattcgcagcgcatcgccttctatcgccttcttgacgagttcttctgaggccatctaggccatgagtaagtctgacggaacggaaagttgtcggttaccagcaacgtttcgccctgttggcctcaaaagttcgagtccgttattggtatttccataccaactcaaacgggatataatgtgacatgtaacatttctcgattgaggaacgacaatgacagtaccggtcaaagcgcgtgttcaaaagtatcgcgacgcgctgcgccgctcgggtttgcgtccggttcagatatgggtgccggatacccgccgcccgggctttgcacaagagtgtcgccgccagtgcctgctcgtgacccaggcagacgccgctgatacgcaactccaacgactcatggatgaagccttggcagagattgatggctggcaggcatgatgcgcggcgatttggtaacgatcgttacccagggcgactttggcaaaccaaggccagcgttggtgatccagtccgatctgttcaacgagctcagcagcataaccgtctttcctgtaaccagtaccattgtggatgccccgttgttgcgcgtcacggttgagccaaccccggaaaacggcttgcacaagcgatcacaggtgatggtggacaaaattatgaccgtgcggcgggacaaagtcggtcagatcattggacgtatcgatacgactacgctgacaacgatcgagcgctgcttagctgtcttcttgggaatcgcgaaataaggccatgaaggccttacccatcaccgtgcatcacgccgaccgcttcgccactttgcgacaagaaagcaatctgaacgcgctggcgaaaatggatcggcgctgcccggtctacctgtgaagttcgcgcaaacgtccatcgagacgtacattgccgttggcatcgatctcgacggcgatttcctctggctaccgatcgcgcgcaccgcttacgcgccctcgacgtagtcgagaaaagcgtgattgcgtatgttgcgccaactgagcccgtcggtgcgttgtgaccactcgttgtagaccacgcccaaaaccatcaccccaaacggtgcggaaagtgctactctttcgtcttgccacaacaagaaggagggcgggtggtgatcgaaaccggtgctttgagagccaaagaagaccccattgcctgggtccaacagaaagcagccgaggcgttgcaacgcctagatcaaaagatggcctctcagcccgtgcagatgtacctaccggggttcgatctaggggcctttcccaaccatgtgaaccgctcctcgctctttgcgcctattgcgcgcggtcgccgcaaatttcatcgacaaacgaagatggtcagccgctcggatgctgtgatcgaatacactggagagcagctcgacgaagccgactgcgacctcatgatggcgctcatctggtttgcccagaaaaaaccgttaggggagtgggtgacattgaaccgagcgcagctgttgcggcggatcgggcgcgcgacgggcaagcagaactacgagtggctccatcgcagaatgcgggcgatgaccgaagcgacactctacatcgaagtgcgcaaatccgacggcagcacacgctacaagatcggctacgccgaggcgtttcacctcatcagcggctttgcgttcgatgagaaaagcgacgaatactgctaccaactcgatccccgctgggtacagctcttcagcaaccgcgaatacagcctgatcaacttcgacttgcgattgcagatcaaacggggtcaggacatggcgaaaaccctgcaacgcctcgttgctacttcttccgaccccatccagtcttacgaactcgaatggctcaagagcaaaatggaatacaccggaagaatgcgcgatttcaaagagtcgctctccaaggcgtgcaatgagctgaaacggttgcacatcgtcagtgaatacaagatcactctggacaaaaagaagcaacgggagctgttgaagctctggattcccaaagcgatcacggcataaaagcggtgcgacactgcacgatcagaaagtattttcagttactcaaacaccgttttttgttgaaaaacaacgaattgtcatcggtatagcgtcgcgcacccgagacgaccgacggtgtctggccatcggtatagcgtcgcgctttctccacctcttgaacagtcgttcggcatcggtatagcgtcgcgcctgcatcggtatagcgtcgcgctttttcggtatagcgtcgcgctttttcggtatagcgtcgcgcggttgtcaaaaaatctattattattcaataagttacaagcggtttttgaccgtctactatatttctacttatttctactaggaagcgcctgtggataacttcgctcttttctacacagcccctcagcggcgcaagcgcgccgctgggtagaaaattcctatcgcaacgaactgtcgttcctaaaaataggctactcggtaaaacaaccgtataaatgatgccgcgtgctcggagtcaactccagaacggcatcggtatagtgtcgcacttagcaatgtgcgaatatttcatcgttgagccgacttttggagattggtcatgggagatcctcgggttgtcgaagccttggactcctgttgatagatccagtaatgacctcagaactccatctggatttgttcagaacgctcggttgccgccgggcgttttttattggtgagaatccagtctaga

SEQ ID NO: 2 - DNA, 1314 bp, Laceyella tengchongensis
  source 1..1314: mol_type = genomic DNA
atgaagaaaaccccaatgtatgaagagacatttgtggcgggcgcgaaagaaccattgaaagtcctgcaccatctggcaacaagtgaatttgttaccgattatctattatatgaaggaaatggtgaggttcggattgtcggcaatgtggtggccaaaatcgaagtgctacaagacattgtccgctttcaatatgctggtgacaccacagaagagccggcgaaggacccgctcaaacaagcggagaggtttttgcacacgcttcctttggagcagtggacggcatatggttatgtggggtttgatatttgcaaatattactacaactacttcaaatccagtgcggagccaatcttgtgtatgatcgtgccggagttcgaacttcgtttcacccaaagcggggtttatataaagtcagtcacccagcaagccgaattgatccaaatattggagtcggagattgatttgccaacctatgagcggtatcctctgaaactggactatgctgaccgtgaaacctatcaacaaaaagtccaatgtctcattgacaatatccaacaacggcaacttcataagacgatcctctcccgttcagtcaaggtacatgatcaacttgatcccattctcacttatgcggaggggacaaacgtcaacaacagcgtgcgttcgtattgccttaaactgggaggcgcaaaagtggtgggcttcagccctgagatcctcatggccgtcgatcgcgagagatttgtgctcaccaatccacttgccgggacgcgcccgcgcggggacacacctgaacgggatcgacaattgcacgatgagttattcaccgatgcaaaagaggtgaaagaacacgctttgtctatctggttggcgcaggatgagattcggagcgtgtgcgagccagatacggttcgggtgctggattttatgcaagtcaaacgataccgctgcgttcagcatttgtcttcacgggttggggggacgatcaaagcggaccggacgtcatgggatgcgttgaaagccttatttcccggcatcaccgtgtcggggattgacaaagcttctgcgttggaatggatttcgcagttggaagaggagccgagaggcatctatgctggagcggtaggatggattgattcaagcgatagagcggatttggcgattgcgatacgctctgttttccaatacggcgatgtcatttcgtttcaagcgggtgccggtatcatgggagaatcgaatcctgagaatgaatacttggagacggttaacaaaatgaacaccatgctgtccacgttggtgctgaaacatgggtga

SEQ ID NO: 3 - protein, 437 aa, Laceyella tengchongensis
MKKTPMYEETFVAGAKEPLKVLHHLATSEFVTDYLLYEGNGEVRIVGNVVAKIEVLQDIVRFQYAGDTTEEPAKDPLKQAERFLHTLPLEQWTAYGYVGFDICKYYYNYFKSSAEPILCMIVPEFELRFTQSGVYIKSVTQQAELIQILESEIDLPTYERYPLKLDYADRETYQQKVQCLIDNIQQRQLHKTILSRSVKVHDQLDPILTYAEGTNVNNSVRSYCLKLGGAKVVGFSPEILMAVDRERFVLTNPLAGTRPRGDTPERDRQLHDELFTDAKEVKEHALSIWLAQDEIRSVCEPDTVRVLDFMQVKRYRCVQHLSSRVGGTIKADRTSWDALKALFPGITVSGIDKASALEWISQLEEEPRGIYAGAVGWIDSSDRADLAIAIRSVFQYGDVISFQAGAGIMGESNPENEYLETVNKMNTMLSTLVLKHG

SEQ ID NO: 4 - DNA, 1458 bp, Alicyclobacillus contaminans
  source 1..1458: mol_type = genomic DNA
atggctggacagcaagtgatggaacaacagaatccgaccgcgaaaacggtgattgaccggctgcgggaagcggcgcactgtgcgctgaataccgcccagcatccgcattgcggctggattgtcaccgcgtcgtttcaacgcgcggtgtcgcgcgagcggctgcggcagctggccggtgcggatccggaagacagtgaacgcatgtactgggcgttgcccggtgcttccgctgcatatttggcattgggacgggcgctggtgatcacaggcgctggatccggacgggtggaagggctgcgtcggcagatggacgcgtacgccatccattccgccgatgctgcggacgttcggcaagccgcagccgatgtgcgctggttcggggggatgtcgtttgctccgaagcggccatcgcaaatgtgggaagggtggcctgaagcgaagttcgtgctcccccacatcgtagtggaatggcaaggtcaggacaccgcgcgggtggttgcaaccgttgccattcacacggcggacgaactggagacgcagttggagggcgttcgccgagagctgcggtggctcgaacggggggcagcggcgtccggaatccatgggaggaaagaacccgtgcctccgtgtcgaccgatggcggaggccgcttggtgtgcgcaggtgtcgagcagtgcggccgagattcgcagcgggcaatacgaaaaagtggtcttagctcggtatgaggcggtgcatggcatacaccggccgctggccgatgtattggcggagctcgaaggcaagtatcccgacagtcaggtgttcgccgtctggcacagtggacagtgctttctcggggcgagccccgagcggctggtctcggtgtccggggagacggtcgatgtggactgtttggccggtacggaggcgcgcggccgcactgccgacgaggatgaacacttggcagcacagttgttggagagtgccaagaatcgcctggaacacgaggtggttcgggcgtggattgtggaacagttgcaaaccgcagatgtcctggatctcacttggccaccgacaccgcaggtgaagcgcctggccaacgtgcagcacttgcatacgcccatccggggacgacggcgggagcagcagtcggtgctcgatttggtggacgagcttcatcccacgcctgccgtggccggtcggccacgcgagaaggcgctcgctgtgattgccgagcgcgagtctttggaacgcggttggtacgcgggccccgtggggtggatgaacggccgtggcgaaggtcaattcgcggtcgcgctgcgcagcgctttggtgcggggcgacacggcgtacgtgttcgcaggcgccggcatcatgggggattcaaatccagcccttgagtgggaggagacgtggatgaaaatgcgggcggttcgaactgcgctgctgccgctcgaagggaggtacagcccgtga

SEQ ID NO: 5 - protein, 485 aa, Alicyclobacillus contaminans
MAGQQVMEQQNPTAKTVIDRLREAAHCALNTAQHPHCGWIVTASFQRAVSRERLRQLAGADPEDSERMYWALPGASAAYLALGRALVITGAGSGRVEGLRRQMDAYAIHSADAADVRQAAADVRWFGGMSFAPKRPSQMWEGWPEAKFVLPHIVVEWQGQDTARVVATVAIHTADELETQLEGVRRELRWLERGAAASGIHGRKEPVPPCRPMAEAAWCAQVSSSAAEIRSGQYEKVVLARYEAVHGIHRPLADVLAELEGKYPDSQVFAVWHSGQCFLGASPERLVSVSGETVDVDCLAGTEARGRTADEDEHLAAQLLESAKNRLEHEVVRAWIVEQLQTADVLDLTWPPTPQVKRLANVQHLHTPIRGRRREQQSVLDLVDELHPTPAVAGRPREKALAVIAERESLERGWYAGPVGWMNGRGEGQFAVALRSALVRGDTAYVFAGAGIMGDSNPALEWEETWMKMRAVRTALLPLEGRYSP

SEQ ID NO: 6 - DNA, 306 bp, Pseudomonas aeruginosa
  source 1..306: mol_type = genomic DNA
atgaaaactcccgaagactgcaccggcctggcggacatccgcgaggccatcgaccggatcgacctggatatcgtccaggccctcggccgccgcatggactacgtcaaggcggcgtcgcgcttcaaggccagcgaggcggcgattccggcgcccgagcgggtcgccgcgatgctccccgagcgcgcccgctgggccgaggagaacggactcgacgcgcccttcgtcgagggactgttcgcgcagatcatccactggtacatcgccgagcagatcaagtactggcgccagacacggggtgccgcatga

SEQ ID NO: 7 - protein, 101 aa, Pseudomonas aeruginosa
MKTPEDCTGLADIREAIDRIDLDIVQALGRRMDYVKAASRFKASEAAIPAPERVAAMLPERARWAEENGLDAPFVEGLFAQIIHWYIAEQIKYWRQTRGAA

SEQ ID NO: 8 - DNA, 20 bp, synthetic construct
  source 1..20: mol_type = other DNA
gaattcgagctccgtcgaca

SEQ ID NO: 9 - DNA, 20 bp, synthetic construct
  source 1..20: mol_type = other DNA
atgcgtttctcctccagatc

SEQ ID NO: 10 - DNA, 1305 bp, Klebsiella pneumoniae
  source 1..1305: mol_type = genomic DNA
atgaaaatcagtgaatttttacacctggcgttaccagaggaacaatggctgccgacgatttctggcgttttacgccagttcgcagaagaagagtgttatgtctatgagcgtcaaccctgttggtatttaggcaaagggtgcctggcacggttgcacattaatgccgacggaacgcaggcgacatttattgatggtgccggggagcaacaatgggcggtggattccattaccgactgcgcgcgtcgttttatggcacatcctcaggtcaaaggacgtcgggtttatggacaggttgggttcaactttgcggcgcatgcgcgggggattgcctttaacgccggggagtggccgctgctgacgttaaccgttccccgtgaagaacttatttttgaaaagggaaatgtcaccgtttatgcggactccgccgacgggggccgacgtttgtgtgagtgggtaaaagaggccagtacaacgacgcagaacgcaccactggcggtggataccgccctcaatggcgaggcgtataaacaacaggttgcacgcgccgttgcggagatccgccgtggcgagtatgtcaaagtgattgtctcgcgcgctattcccctgccatcgcggattgatatgcccgccacgctgttatacgggcggcaggcaaatacacctgtgcgctcgtttatgttccgtcaggaaggacgcgaagcgctgggctttagcccggaactggtgatgtcagtgacgggcaataaagtggtcactgaaccgcttgcgggcacccgcgatcgcatgggaaacccggagcataataaggcgaaagaggcagaactgctgcacgacagtaaagaggtgcttgagcatatcctttctgtcaaagaagcgattgctgaactggaggccgtttgcctgctgggcagcgtggtggttgaagatttaatgtcggttcgccagcgcggcagcgttcagcatctggggtccggcgtgagcggtcagcttgcggaaaacaaggatgcctgggatgcgtttaccgtgctgtttccgtcgattaccgcctcaggtatccctaaaaacgctgccctgaacgcgattatgcaaattgagaagacgccgcgagagctctattccggcgcaattctgctgctggacgatatgcgcttcgatgcggcgctagttctgcgttccgtatttcaggacagccagcgctgctggatacaagcgggggcgggaatcatcgcgcaatctacaccggaacgcgaactgacggaaaccagggagaaattagcgagcattgcgccctatttaatggtgtag

SEQ ID NO: 11 - DNA, 42 bp, synthetic construct
  source 1..42: mol_type = other DNA
ctggaggagaaacgcatatgaagaaaaccccaatgtatgaag

SEQ ID NO: 12 - DNA, 44 bp, synthetic construct
  source 1..44: mol_type = other DNA
gtcgacggagctcgaattctcacccatgtttcagcaccaacgtg

SEQ ID NO: 13 - DNA, 44 bp, synthetic construct
  source 1..44: mol_type = other DNA
gatctggaggagaaacgcatatgaaaatcagtgaatttttacac

SEQ ID NO: 14 - DNA, 43 bp, synthetic construct
  source 1..43: mol_type = other DNA
cgacggagctcgaattcctacaccattaaatagggcgcaatgc

SEQ ID NO: 15 - DNA, 41 bp, synthetic construct
  source 1..41: mol_type = other DNA
gatctggaggagaaacgcatatggctggacagcaagtgatg

SEQ ID NO: 16 - DNA, 44 bp, synthetic construct
  source 1..44: mol_type = other DNA
gtcgacggagctcgaattctcacgggctgtacctcccttcgagc

SEQ ID NO: 17 - DNA, 43 bp, synthetic construct
  source 1..43: mol_type = other DNA
gatctggaggagaaacgcatatgaaaactcccgaagactgcac

SEQ ID NO: 18 - DNA, 43 bp, synthetic construct
  source 1..43: mol_type = other DNA
gtcgacggagctcgaattctcatgcggcaccccgtgtctggcg

SEQ ID NO: 19 - DNA, 35 bp, synthetic construct
  source 1..35: mol_type = other DNA
ggctcgtataatgtgtggaattgtgagcggataac

SEQ ID NO: 20 - DNA, 43 bp, synthetic construct
  source 1..43: mol_type = other DNA
atgcgatactcctcctcacgggctgtacctcccttcgagcggc

SEQ ID NO: 21 - DNA, 44 bp, synthetic construct
  source 1..44: mol_type = other DNA
ccgtgaggaggagtatcgcatatgaaaactcccgaagactgcac

SEQ ID NO: 22 - DNA, 35 bp, synthetic construct
  source 1..35: mol_type = other DNA
ccggcggatttgtcctactcaggagagcgttcacc